European Patent Specification EP 3 408 380 B1, published December 13, 2023. Title: AAV-based conditional expression system. Applicant: Sirion Biotech GmbH Ludwig-Maximilians-Universität München. The sequence listing filed with the application follows.

SEQUENCE LISTING (10 sequences)

SEQ ID NO: 1 - DNA, 8977 bp, Artificial Sequence
  Conditional expression system
atcgataagcttctagagatctgggccactccctctctgcgcgctcgctcgctcactgaggccgggcgaccaaaggtcgcccgacgcccgggctttgcccgggcggcctcagtgagcgagcgagcgcgcagagagggagtggccaactccatcactaggggttcctggaggggtggagtcgtgacgtgaattacgtcatagggttagggaggtcctgtattagaggtcacgtgagtgttttgcgacattttgcgacaccatgtggtcacgctgggtatttaagcccgagtgagcacgcagggtctccattttgaagcgggaggtttgaacgcgcagccgccatgccggggttttacgagattgtgattaaggtccccagcgaccttgacgggcatctgcccggcatttctgacagctttgtgaactgggtggccgagaaggaatgggagttgccgccagattctgacatggatctgaatctgattgagcaggcacccctgaccgtggccgagaagctgcagcgcgactttctgacggaatggcgccgtgtgagtaaggccccggaggcccttttctttgtgcaatttgagaagggagagagctacttccacatgcacgtgctcgtggaaaccaccggggtgaaatccatggttttgggacgtttcctgagtcagattcgcgaaaaactgattcagagaatttaccgcgggatcgagccgactttgccaaactggttcgcggtcacaaagaccagaaatggcgccggaggcgggaacaaggtggtggatgagtgctacatccccaattacttgctccccaaaacccagcctgagctccagtgggcgtggactaatatggaacagtatttaagcgcctgtttgaatctcacggagcgtaaacggttggtggcgcagcatctgacgcacgtgtcgcagacgcaggagcagaacaaagagaatcagaatcccaattctgatgcgccggtgatcagatcaaaaacttcagccaggtacatggagctggtcgggtggctcgtggacaaggggattacctcggagaagcagtggatccaggaggaccaggcctcatacatctccttcaatgcggcctccaactcgcggtcccaaatcaaggctgccttggacaatgcgggaaagattatgagcctgactaaaaccgcccccgactacctggtgggccagcagcccgtggaggacatttccagcaatcggatttataaaattttggaactaaacgggtacgatccccaatatgcggcttccgtctttctgggatgggccacgaaaaagttcggcaagaggaacaccatctggctgtttgggcctgcaactaccgggaagaccaacatcgcggaggccatagcccacactgtgcccttctacgggtgcgtaaactggaccaatgagaactttcccttcaacgactgtgtcgacaagatggtgatctggtgggaggaggggaagatgaccgccaaggtcgtggagtcggccaaagccattctcggaggaagcaaggtgcgcgtggaccagaaatgcaagtcctcggcccagatagacccgactcccgtgatcgtcacctccaacaccaacatgtgcgccgtgattgacgggaactcaacgaccttcgaacaccagcagccgttgcaagaccggatgttcaaatttgaactcacccgccgtctggatcatgactttgggaaggtcaccaagcaggaagtcaaagactttttccggtgggcaaaggatcacgtggttgaggtggagcatgaattctacgtcaaaaagggtggagccaagaaaagacccgcccccagtgacgcagatataagtgagcccaaacgggtgcgcgagtcagttgcgcagccatcgacgtcagacgcggaagcttcgatcaactacgcagacaggtaccaaaacaaatgttctcgtcacgtgggcatgaatctgatgctgtttccctgcagacaatgcgagagaatgaatcagaattcaaatatctgcttcactcacggacagaaagactgtttagagtgctttcccgtgtcagaatctcaacccgtttctgtcgtcaaaaaggcgtatcagaaactgtgctacattcatcatatcatgggaaaggtgccagacgcttgcactgcctgcgatctggtcaatgtggatttggatgactgcatctttgaacaataaatgatttaaatcaggtatggctgccgatggttatcttccagattggctcgaggacactctctctgagctagcttcgtacggatcctcggatccagccaccatgggagtcaaagttctgtttgccctgatctgcatcgctgtggccgaggccaagcccaccgagaacaacgaagacttcaacatcgtggccgtggccagcaacttcgcgaccacggatctcgatgctgaccgcgggaagttgcccggcaagaagctgccgctggaggtgctcaaagagatggaagccaatgcccggaaagctggctgcaccaggggctgtctgatctgcctgtcccacatcaagtgcacgcccaagatgaagaagttcatcccaggacgctgccacacctacgaaggcgacaaagagtccgcacagggcggcataggcgaggcgatcgtcgacattcctgagattcctgggttcaaggacttggagcccatggagcagttcatcgcacaggtcgatctgtgtgtggactgcacaactggctgcctcaaagggcttgccaacgtgcagtgttctgacctgctcaagaagtggctgccgcaacgctgtgcgacctttgccagcaagatccagggccaggtggacaagatcaagggggccggtggtgactaagcggccgcgtgtggaaagtccccaggctccccagcaggcagaagtatgcaaagcatgcatctcaattagtcagcaaccaggtgtggaaagtccccaggctccccagcaggcagaagtatgcaaagcatgcatctcaattagtcagcaaccatagtcccgcccctaactccgcccatcccgcccctaactccgcccagttccgcccattctccgccccatggctgactaattttttttatttatgcagaggccgaggccgcctcggcctctgagctattccagaagtagtgaggaggcttttttggaggcctaggcttttgcaaaaagcttccatgaaaaagcctgaactcaccgcgacgtctgtcgagaagtttctgatcgaaaagttcgacagcgtctccgacctgatgcagctctcggagggcgaagaatctcgtgctttcagcttcgatgtaggagggcgtggatatgtcctgcgggtaaatagctgcgccgatggtttctacaaagatcgttatgtttatcggcactttgcatcggccgcgctcccgattccggaagtgcttgacattggggaattcagcgagagcctgacctattgcatctcccgccgtgcacagggtgtcacgttgcaagacctgcctgaaaccgaactgcccgctgttctgcagccggtcgcggaggccatggatgcgatcgctgcggccgatcttagccagacgagcgggttcggcccattcggaccgcaaggaatcggtcaatacactacatggcgtgatttcatatgcgcgattgctgatccccatgtgtatcactggcaaactgtgatggacgacaccgtcagtgcgtccgtcgcgcaggctctcgatgagctgatgctttgggccgaggactgccccgaagtccggcacctcgtgcacgcggatttcggctccaacaatgtcctgacggacaatggccgcataacagcggtcattgactggagcgaggcgatgttcggggattcccaatacgaggtcgccaacatcttcttctggaggccgtggttggcttgtatggagcagcagacgcgctacttcgagcggaggcatccggagcttgcaggatcgccgcggctccgggcgtatatgctccgcattggtcttgaccaactctatcagagcttggttgacggcaatttcgatgatgcagcttgggcgcagggtcgatgcgacgcaatcgtccgatccggagccgggactgtcgggcgtacacaaatcgcccgcagaagcgcggccgtctggaccgatggctgtgtagaagtactcgccgatagtggaaaccgacgccccagcactcgtccgagggcaaaggaatagagttctagaggatcataatcagccataccacagggcccatctgggcaaagattccacacacggacggacattttcacccctctcccctcatgggtggattcggacttaaacaccctcctccacagattctcatcaagaacaccccggtacctgcgaatccttcgaccaccttcagtgcggcaaagtttgcttccttcatcacacagtactccacgggacacggtcagcgtggagatcgagtgggagctgcagaaggaaaacagcaaacgctggaatcccgaaattcagtacacttccaactacaacaagtctgttaatcgtggacttaccgtggatactaatggcgtgtattcagagcctcgccccattggcaccagatacctgactcgtaatctgtaattgcttgttaatcaataaaccgtttaattcgtttcagttgaactttggtctctgcgtatttctttcttatctagtttccatggctacgtagataagtagcatggcgggttaatcattaactacaaggaacccctagtgatggagttggccactccctctctgcgcgctcgctcgctcactgaggccgggcgaccaaaggtcgcccgacgcccgggctttgcccgggcggcctcagtgagcgagcgagcgcgcagagagggacagatcttccatacctaccagttctgcgcctgcagcaatggcaacaacgttgcccggatccggtcgcgcgaattcttgaagacgaaagggcctcgtgatacgcctatttttataggttaatgtcatgataataatggtttcttagacgtcaggtggcacttttcggggaaatgtgcgcggaacccctatttgtttatttttctaaatacattcaaatatgtatccgctcatgagacaataaccctgataaatgcttcaataatattgaaaaaggaagagtatgagtattcaacatttccgtgtcgcccttattcccttttttgcggcattttgccttcctgtttttgctcacccagaaacgctggtgaaagtaaaagatgctgaagatcagttgggtgcacgagtgggttacatcgaactggatctcaacagcggtaagatccttgagagttttcgccccgaagaacgttttccaatgatgagcacttttaaagttctgctatgtggcgcggtattatcccgtgttgacgccgggcaagagcaactcggtcgccgcatacactattctcagaatgacttggttgagtactcaccagtcacagaaaagcatcttacggatggcatgacagtaagagaattatgcagtgctgccataaccatgagtgataacactgcggccaacttacttctgacaacgatcggaggaccgaaggagctaaccgcttttttgcacaacatgggggatcatgtaactcgccttgatcgttgggaaccggagctgaatgaagccataccaaacgacgagcgtgacaccacgatgcctgcagcaatggcaacaacgttgcgcaaactattaactggcgaactacttactctagcttcccggcaacaattaatagactggatggaggcggataaagttgcaggaccacttctgcgctcggcccttccggctggctggtttattgctgataaatctggagccggtgagcgtgggtctcgcggtatcattgcagcactggggccagatggtaagccctcccgtatcgtagttatctacacgacggggagtcaggcaactatggatgaacgaaatagacagatcgctgagataggtgcctcactgattaagcattggtaactgtcagaccaagtttactcatatatactttagattgatttaaaacttcatttttaatttaaaaggatctaggtgaagatcctttttgataatctcatgaccaaaatcccttaacgtgagttttcgttccactgagcgtcagaccccgtagaaaagatcaaaggatcttcttgagatcctttttttctgcgcgtaatctgctgcttgcaaacaaaaaaaccaccgctaccagcggtggtttgtttgccggatcaagagctaccaactctttttccgaaggtaactggcttcagcagagcgcagataccaaatactgtccttctagtgtagccgtagttaggccaccacttcaagaactctgtagcaccgcctacatacctcgctctgctaatcctgttaccagtggctgctgccagtggcgataagtcgtgtcttaccgggttggactcaagacgatagttaccggataaggcgcagcggtcgggctgaacggggggttcgtgcacacagcccagcttggagcgaacgacctacaccgaactgagatacctacagcgtgagctatgagaaagcgccacgcttcccgaagggagaaaggcggacaggtatccggtaagcggcagggtcggaacaggagagcgcacgagggagcttccagggggaaacgcctggtatctttatagtcctgtcgggtttcgccacctctgacttgagcgtcgatttttgtgatgctcgtcaggggggcggagcctatggaaaaacgccagcaacgcggcctttttacggttcctggccttttgctggccttttgctcacatgttctttcctgcgttatcccctgattctgtggataaccgtattaccgcctttgagtgagctgataccgctcgccgcagccgaacgaccgagcgcagcgagtcagtgagcgaggaagcggaagagcgcctgatgcggtattttctccttacgcatctgtgcggtatttcacaccgcatatggtgcactctcagtacaatctgctctgatgccgcatagttaagccagtatacactccgctatcgctacgtgactgggtcatggctgcgccccgacacccgccaacacccgctgacgcgccctgacgggcttgtctgctcccggcatccgcttacagacaagctgtgaccgtctccgggagctgcatgtgtcagaggttttcaccgtcatcaccgaaacgcgcgaggcagctgcggtaaagctcatcagcgtggtcgtgaagcgattcacagatgtctgcctgttcatccgcgtccagctcgttgagtttctccagaagcgttaatgtctggcttctgataaagcgggccatgttaagggcggttttttcctgtttggtcactgatgcctccgtgtaagggggatttctgttcatgggggtaatgataccgatgaaacgagagaggatgctcacgatacgggttactgatgatgaacatgcccggttactggaacgttgtgagggtaaacaactggcggtatggatgcggcgggaccagagaaaaatcactcagggtcaatgccagcgcttcgttaatacagatgtaggtgttccacagggtagccagcagcatcctgcgatgcagatccggaacataatggtgcagggcgctgacttccgcgtttccagactttacgaaacacggaaaccgaagaccattcatgttgttgctcaggtcgcagacgttttgcagcagcagtcgcttcacgttcgctcgcgtatcggtgattcattctgctaaccagtaaggcaaccccgccagcctagccgggtcctcaacgacaggagcacgatcatgcgcacccgtggccaggacccaacgctgcccgagatgcgccgcgtgcggctgctggagatggcggacgcgatggatatgttctgccaagggttggtttgcgcattcacagttctccgcaagaattgattggctccaattcttggagtggtgaatccgttagcgaggtgccgccggcttccattcaggtcgaggtggcccggctccatgcaccgcgacgcaacgcggggaggcagacaaggtatagggcggcgcctacaatccatgccaacccgttccatgtgctcgccgaggcggcataaatcgccgtgacgatcagcggtccagtgatcgaagttaggctggtaagagccgcgagcgatccttgaagctgtccctgatggtcgtcatctacctgcctggacagcatggcctgcaacgcgggcatcccgatgccgccggaagcgagaagaatcataatggggaaggccatccagcctcgcgtcgcgaacgccagcaagacgtagcccagcgcgtcggccgccatgccggcgataatggcctgcttctcgccgaaacgtttggtggcgggaccagtgacgaaggcttgagcgagggcgtgcaagattccgaataccgcaagcgacaggccgatcatcgtcgcgctccagcgaaagcggtcctcgccgaaaatgacccagagcgctgccggcacctgtcctacgagttgcatgataaagaagacagtcataagtgcggcgacgatagtcatgccccgcgcccaccggaaggagctgactgggttgaaggctctcaagggcatcggtcgacgctctcccttatgcgactcctgcattaggaagcagcccagtagtaggttgaggccgttgagcaccgccgccgcaaggaatggtgcatgcaaggagatggcgcccaacagtcccccggccacggggcctgccaccatacccacgccgaaacaagcgctcatgagcccgaagtggcgagcccgatcttccccatcggtgatgtcggcgatataggcgccagcaaccgcacctgtggcgccggtgatgccggccacgatgcgtccggcgtagagctctagagctctagagaattctcatgtttgacagcttatc

SEQ ID NO: 2 - DNA, 33 bp, Artificial Sequence
  Primer
gtgtaggcctcggatccagccaccatgggagtc

SEQ ID NO: 3 - DNA, 22 bp, Artificial Sequence
  Primer
ccatagagcccaccgcatcccc

SEQ ID NO: 4 - DNA, 20 bp, Artificial Sequence
  Primer
tggtatcgtggaaggactca

SEQ ID NO: 5 - DNA, 20 bp, Artificial Sequence
  Primer
ccagtagaggcagggatgat

SEQ ID NO: 6 - protein, 536 aa, Adeno-associated virus - 2
  Rep 68
MPGFYEIVIKVPSDLDEHLPGISDSFVNWVAEKEWELPPDSDMDLNLIEQAPLTVAEKLQRDFLTEWRRVSKAPEALFFVQFEKGESYFHMHVLVETTGVKSMVLGRFLSQIREKLIQRIYRGIEPTLPNWFAVTKTRNGAGGGNKVVDECYIPNYLLPKTQPELQWAWTNMEQYLSACLNLTERKRLVAQHLTHVSQTQEQNKENQNPNSDAPVIRSKTSARYMELVGWLVDKGITSEKQWIQEDQASYISFNAASNSRSQIKAALDNAGKIMSLTKTAPDYLVGQQPVEDISSNRIYKILELNGYDPQYAASVFLGWATKKFGKRNTIWLFGPATTGKTNIAEAIAHTVPFYGCVNWTNENFPFNDCVDKMVIWWEEGKMTAKVVESAKAILGGSKVRVDQKCKSSAQIDPTPVIVTSNTNMCAVIDGNSTTFEHQQPLQDRMFKFELTRRLDHDFGKVTKQEVKDFFRWAKDHVVEVEHEFYVKKGGAKKRPAPSDADISEPKRVRESVAQPSTSDAEASINYADRLARGHSL

SEQ ID NO: 7 - protein, 621 aa, Adeno-associated virus - 2
  Rep 78
MPGFYEIVIKVPSDLDEHLPGISDSFVNWVAEKEWELPPDSDMDLNLIEQAPLTVAEKLQRDFLTEWRRVSKAPEALFFVQFEKGESYFHMHVLVETTGVKSMVLGRFLSQIREKLIQRIYRGIEPTLPNWFAVTKTRNGAGGGNKVVDECYIPNYLLPKTQPELQWAWTNMEQYLSACLNLTERKRLVAQHLTHVSQTQEQNKENQNPNSDAPVIRSKTSARYMELVGWLVDKGITSEKQWIQEDQASYISFNAASNSRSQIKAALDNAGKIMSLTKTAPDYLVGQQPVEDISSNRIYKILELNGYDPQYAASVFLGWATKKFGKRNTIWLFGPATTGKTNIAEAIAHTVPFYGCVNWTNENFPFNDCVDKMVIWWEEGKMTAKVVESAKAILGGSKVRVDQKCKSSAQIDPTPVIVTSNTNMCAVIDGNSTTFEHQQPLQDRMFKFELTRRLDHDFGKVTKQEVKDFFRWAKDHVVEVEHEFYVKKGGAKKRPAPSDADISEPKRVRESVAQPSTSDAEASINYADRYQNKCSRHVGMNLMLFPCRQCERMNQNSNICFTHGQKDCLECFPVSESQPVSVVKKAYQKLCYIHHIMGKVPDACTACDLVNVDLDDCIFEQ

SEQ ID NO: 8 - protein, 312 aa, Adeno-associated virus - 2
  Rep 40
MELVGWLVDKGITSEKQWIQEDQASYISFNAASNSRSQIKAALDNAGKIMSLTKTAPDYLVGQQPVEDISSNRIYKILELNGYDPQYAASVFLGWATKKFGKRNTIWLFGPATTGKTNIAEAIAHTVPFYGCVNWTNENFPFNDCVDKMVIWWEEGKMTAKVVESAKAILGGSKVRVDQKCKSSAQIDPTPVIVTSNTNMCAVIDGNSTTFEHQQPLQDRMFKFELTRRLDHDFGKVTKQEVKDFFRWAKDHVVEVEHEFYVKKGGAKKRPAPSDADISEPKRVRESVAQPSTSDAEASINYADRLARGHSL

SEQ ID NO: 9 - protein, 397 aa, Adeno-associated virus - 2
  Rep 52
MELVGWLVDKGITSEKQWIQEDQASYISFNAASNSRSQIKAALDNAGKIMSLTKTAPDYLVGQQPVEDISSNRIYKILELNGYDPQYAASVFLGWATKKFGKRNTIWLFGPATTGKTNIAEAIAHTVPFYGCVNWTNENFPFNDCVDKMVIWWEEGKMTAKVVESAKAILGGSKVRVDQKCKSSAQIDPTPVIVTSNTNMCAVIDGNSTTFEHQQPLQDRMFKFELTRRLDHDFGKVTKQEVKDFFRWAKDHVVEVEHEFYVKKGGAKKRPAPSDADISEPKRVRESVAQPSTSDAEASINYADRYQNKCSRHVGMNLMLFPCRQCERMNQNSNICFTHGQKDCLECFPVSESQPVSVVKKAYQKLCYIHHIMGKVPDACTACDLVNVDLDDCIFEQ

SEQ ID NO: 10 - DNA, 4854 bp, Artificial Sequence
  Conditional expression system
tgggccactccctctctgcgcgctcgctcgctcactgaggccgggcgaccaaaggtcgcccgacgcccgggctttgcccgggcggcctcagtgagcgagcgagcgcgcagagagggagtggccaactccatcactaggggttcctggaggggtggagtcgtgacgtgaattacgtcatagggttagggaggtcctgtattagaggtcacgtgagtgttttgcgacattttgcgacaccatgtggtcacgctgggtatttaagcccgagtgagcacgcagggtctccattttgaagcgggaggtttgaacgcgcagccgccatgccggggttttacgagattgtgattaaggtccccagcgaccttgacgggcatctgcccggcatttctgacagctttgtgaactgggtggccgagaaggaatgggagttgccgccagattctgacatggatctgaatctgattgagcaggcacccctgaccgtggccgagaagctgcagcgcgactttctgacggaatggcgccgtgtgagtaaggccccggaggcccttttctttgtgcaatttgagaagggagagagctacttccacatgcacgtgctcgtggaaaccaccggggtgaaatccatggttttgggacgtttcctgagtcagattcgcgaaaaactgattcagagaatttaccgcgggatcgagccgactttgccaaactggttcgcggtcacaaagaccagaaatggcgccggaggcgggaacaaggtggtggatgagtgctacatccccaattacttgctccccaaaacccagcctgagctccagtgggcgtggactaatatggaacagtatttaagcgcctgtttgaatctcacggagcgtaaacggttggtggcgcagcatctgacgcacgtgtcgcagacgcaggagcagaacaaagagaatcagaatcccaattctgatgcgccggtgatcagatcaaaaacttcagccaggtacatggagctggtcgggtggctcgtggacaaggggattacctcggagaagcagtggatccaggaggaccaggcctcatacatctccttcaatgcggcctccaactcgcggtcccaaatcaaggctgccttggacaatgcgggaaagattatgagcctgactaaaaccgcccccgactacctggtgggccagcagcccgtggaggacatttccagcaatcggatttataaaattttggaactaaacgggtacgatccccaatatgcggcttccgtctttctgggatgggccacgaaaaagttcggcaagaggaacaccatctggctgtttgggcctgcaactaccgggaagaccaacatcgcggaggccatagcccacactgtgcccttctacgggtgcgtaaactggaccaatgagaactttcccttcaacgactgtgtcgacaagatggtgatctggtgggaggaggggaagatgaccgccaaggtcgtggagtcggccaaagccattctcggaggaagcaaggtgcgcgtggaccagaaatgcaagtcctcggcccagatagacccgactcccgtgatcgtcacctccaacaccaacatgtgcgccgtgattgacgggaactcaacgaccttcgaacaccagcagccgttgcaagaccggatgttcaaatttgaactcacccgccgtctggatcatgactttgggaaggtcaccaagcaggaagtcaaagactttttccggtgggcaaaggatcacgtggttgaggtggagcatgaattctacgtcaaaaagggtggagccaagaaaagacccgcccccagtgacgcagatataagtgagcccaaacgggtgcgcgagtcagttgcgcagccatcgacgtcagacgcggaagcttcgatcaactacgcagacaggtaccaaaacaaatgttctcgtcacgtgggcatgaatctgatgctgtttccctgcagacaatgcgagagaatgaatcagaattcaaatatctgcttcactcacggacagaaagactgtttagagtgctttcccgtgtcagaatctcaacccgtttctgtcgtcaaaaaggcgtatcagaaactgtgctacattcatcatatcatgggaaaggtgccagacgcttgcactgcctgcgatctggtcaatgtggatttggatgactgcatctttgaacaataaatgatttaaatcaggtatggctgccgatggttatcttccagattggctcgaggacactctctctgagctagcttcgtacggatcctcggatccagccaccatgggagtcaaagttctgtttgccctgatctgcatcgctgtggccgaggccaagcccaccgagaacaacgaagacttcaacatcgtggccgtggccagcaacttcgcgaccacggatctcgatgctgaccgcgggaagttgcccggcaagaagctgccgctggaggtgctcaaagagatggaagccaatgcccggaaagctggctgcaccaggggctgtctgatctgcctgtcccacatcaagtgcacgcccaagatgaagaagttcatcccaggacgctgccacacctacgaaggcgacaaagagtccgcacagggcggcataggcgaggcgatcgtcgacattcctgagattcctgggttcaaggacttggagcccatggagcagttcatcgcacaggtcgatctgtgtgtggactgcacaactggctgcctcaaagggcttgccaacgtgcagtgttctgacctgctcaagaagtggctgccgcaacgctgtgcgacctttgccagcaagatccagggccaggtggacaagatcaagggggccggtggtgactaagcggccgcgtgtggaaagtccccaggctccccagcaggcagaagtatgcaaagcatgcatctcaattagtcagcaaccaggtgtggaaagtccccaggctccccagcaggcagaagtatgcaaagcatgcatctcaattagtcagcaaccatagtcccgcccctaactccgcccatcccgcccctaactccgcccagttccgcccattctccgccccatggctgactaattttttttatttatgcagaggccgaggccgcctcggcctctgagctattccagaagtagtgaggaggcttttttggaggcctaggcttttgcaaaaagcttccatgaaaaagcctgaactcaccgcgacgtctgtcgagaagtttctgatcgaaaagttcgacagcgtctccgacctgatgcagctctcggagggcgaagaatctcgtgctttcagcttcgatgtaggagggcgtggatatgtcctgcgggtaaatagctgcgccgatggtttctacaaagatcgttatgtttatcggcactttgcatcggccgcgctcccgattccggaagtgcttgacattggggaattcagcgagagcctgacctattgcatctcccgccgtgcacagggtgtcacgttgcaagacctgcctgaaaccgaactgcccgctgttctgcagccggtcgcggaggccatggatgcgatcgctgcggccgatcttagccagacgagcgggttcggcccattcggaccgcaaggaatcggtcaatacactacatggcgtgatttcatatgcgcgattgctgatccccatgtgtatcactggcaaactgtgatggacgacaccgtcagtgcgtccgtcgcgcaggctctcgatgagctgatgctttgggccgaggactgccccgaagtccggcacctcgtgcacgcggatttcggctccaacaatgtcctgacggacaatggccgcataacagcggtcattgactggagcgaggcgatgttcggggattcccaatacgaggtcgccaacatcttcttctggaggccgtggttggcttgtatggagcagcagacgcgctacttcgagcggaggcatccggagcttgcaggatcgccgcggctccgggcgtatatgctccgcattggtcttgaccaactctatcagagcttggttgacggcaatttcgatgatgcagcttgggcgcagggtcgatgcgacgcaatcgtccgatccggagccgggactgtcgggcgtacacaaatcgcccgcagaagcgcggccgtctggaccgatggctgtgtagaagtactcgccgatagtggaaaccgacgccccagcactcgtccgagggcaaaggaatagagttctagaggatcataatcagccataccacagggcccatctgggcaaagattccacacacggacggacattttcacccctctcccctcatgggtggattcggacttaaacaccctcctccacagattctcatcaagaacaccccggtacctgcgaatccttcgaccaccttcagtgcggcaaagtttgcttccttcatcacacagtactccacgggacacggtcagcgtggagatcgagtgggagctgcagaaggaaaacagcaaacgctggaatcccgaaattcagtacacttccaactacaacaagtctgttaatcgtggacttaccgtggatactaatggcgtgtattcagagcctcgccccattggcaccagatacctgactcgtaatctgtaattgcttgttaatcaataaaccgtttaattcgtttcagttgaactttggtctctgcgtatttctttcttatctagtttccatggctacgtagataagtagcatggcgggttaatcattaactacaaggaacccctagtgatggagttggccactccctctctgcgcgctcgctcgctcactgaggccgggcgaccaaaggtcgcccgacgcccgggctttgcccgggcggcctcagtgagcgagcgagcgcgca